European Patent Specification EP 3 687 559 B1, published November 12, 2025. Title: COMPOSITIONS THAT TARGET TUMOR-ASSOCIATED MACROPHAGES AND METHODS OF USE THEREFOR. Applicant: Sanford Burnhan Institute Teesalu, Tambet Scodeller, Pablo Ruoslahti, Erkki. The sequence listing filed with the application follows.

SEQUENCE LISTING (78 sequences)

SEQ ID NO: 1 - protein, 9 aa, Artificial Sequence
  Synthetic polypeptide
CSPGAKVRC

SEQ ID NO: 2 - protein, 6 aa, Artificial Sequence
  Synthetic polypeptide
GSPGAK

SEQ ID NO: 3 - protein, 9 aa, Artificial Sequence
  Synthetic polypeptide
CGEKRTRGC

SEQ ID NO: 4 - protein, 9 aa, Artificial Sequence
  Synthetic polypeptide
CGNKRTRGC

SEQ ID NO: 5 - protein, 9 aa, Artificial Sequence
  Synthetic polypeptide
CRKQGEAKC

SEQ ID NO: 6 - protein, 6 aa, Artificial Sequence
  Synthetic polypeptide
CSPGAK

SEQ ID NO: 7 - protein, 7 aa, Artificial Sequence
  Synthetic polypeptide
CPMTDNE

SEQ ID NO: 8 - protein, 9 aa, Artificial Sequence
  Synthetic polypeptide
CDSRSRKRC

SEQ ID NO: 9 - protein, 9 aa, Artificial Sequence
  Synthetic polypeptide
CPKGAGSKC

SEQ ID NO: 10 - protein, 9 aa, Artificial Sequence
  Synthetic polypeptide
CRKGTLGRC

SEQ ID NO: 11 - protein, 9 aa, Artificial Sequence
  Synthetic polypeptide
CVKGTVKTC

SEQ ID NO: 12 - protein, 9 aa, Artificial Sequence
  Synthetic polypeptide
CRGTIRGRC

SEQ ID NO: 13 - protein, 9 aa, Artificial Sequence
  Synthetic polypeptide
CLDRRKKPC

SEQ ID NO: 14 - protein, 9 aa, Artificial Sequence
  Synthetic polypeptide
CPARRSNRC

SEQ ID NO: 15 - protein, 9 aa, Artificial Sequence
  Synthetic polypeptide
CKDSAEMRC

SEQ ID NO: 16 - protein, 9 aa, Artificial Sequence
  Synthetic polypeptide
CERSNNVSC

SEQ ID NO: 17 - protein, 9 aa, Artificial Sequence
  Synthetic polypeptide
CGKRAPFRC

SEQ ID NO: 18 - protein, 9 aa, Artificial Sequence
  Synthetic polypeptide
CVSSSSGRC

SEQ ID NO: 19 - protein, 9 aa, Artificial Sequence
  Synthetic polypeptide
CTVAGSGPC

SEQ ID NO: 20 - protein, 9 aa, Artificial Sequence
  Synthetic polypeptide
CIGNSKKKC

SEQ ID NO: 21 - protein, 9 aa, Artificial Sequence
  Synthetic polypeptide
CVRLREKRC

SEQ ID NO: 22 - protein, 9 aa, Artificial Sequence
  Synthetic polypeptide
CRKKSRAQC

SEQ ID NO: 23 - protein, 9 aa, Artificial Sequence
  Synthetic polypeptide
CAANDYSDC

SEQ ID NO: 24 - protein, 9 aa, Artificial Sequence
  Synthetic polypeptide
CLEDDSAKC

SEQ ID NO: 25 - protein, 5 aa, Artificial Sequence
  Synthetic polypeptide
CNDKS

SEQ ID NO: 26 - protein, 9 aa, Artificial Sequence
  Synthetic polypeptide
CVGRKVRGC

SEQ ID NO: 27 - protein, 9 aa, Artificial Sequence
  Synthetic polypeptide
CVDRRESRC

SEQ ID NO: 28 - protein, 9 aa, Artificial Sequence
  Synthetic polypeptide
CRQEEESRC

SEQ ID NO: 29 - protein, 9 aa, Artificial Sequence
  Synthetic polypeptide
CGKTRYSRC

SEQ ID NO: 30 - protein, 8 aa, Artificial Sequence
  Synthetic polypeptide
CIGVSSDC

SEQ ID NO: 31 - protein, 9 aa, Artificial Sequence
  Synthetic polypeptide
CRTLRSKAC

SEQ ID NO: 32 - protein, 9 aa, Artificial Sequence
  Synthetic polypeptide
CRRTRQRSC

SEQ ID NO: 33 - protein, 5 aa, Artificial Sequence
  Synthetic polypeptide
CIGNK

SEQ ID NO: 34 - protein, 9 aa, Artificial Sequence
  Synthetic polypeptide
CVLNESGDC

SEQ ID NO: 35 - protein, 9 aa, Artificial Sequence
  Synthetic polypeptide
CRDKRGSKC

SEQ ID NO: 36 - protein, 9 aa, Artificial Sequence
  Synthetic polypeptide
CKRPNENVC

SEQ ID NO: 37 - protein, 9 aa, Artificial Sequence
  Synthetic polypeptide
CNRRTKIGC

SEQ ID NO: 38 - protein, 9 aa, Artificial Sequence
  Synthetic polypeptide
CSPKMRATC

SEQ ID NO: 39 - protein, 9 aa, Artificial Sequence
  Synthetic polypeptide
CKRTRRREC

SEQ ID NO: 40 - protein, 9 aa, Artificial Sequence
  Synthetic polypeptide
CLSSITPEC

SEQ ID NO: 41 - protein, 7 aa, Artificial Sequence
  Synthetic polypeptide
CVDQDPL

SEQ ID NO: 42 - protein, 9 aa, Artificial Sequence
  Synthetic polypeptide
CRGTRSNRC

SEQ ID NO: 43 - protein, 9 aa, Artificial Sequence
  Synthetic polypeptide
CGPCQEGLC

SEQ ID NO: 44 - protein, 9 aa, Artificial Sequence
  Synthetic polypeptide
CMTLRSRKC

SEQ ID NO: 45 - protein, 9 aa, Artificial Sequence
  Synthetic polypeptide
CSTKTSLKC

SEQ ID NO: 46 - protein, 5 aa, Artificial Sequence
  Synthetic polypeptide
CGDEA

SEQ ID NO: 47 - protein, 9 aa, Artificial Sequence
  Synthetic polypeptide
CTTSTGADC

SEQ ID NO: 48 - protein, 9 aa, Artificial Sequence
  Synthetic polypeptide
CSTLKRRVC

SEQ ID NO: 49 - protein, 9 aa, Artificial Sequence
  Synthetic polypeptide
CRGVAKVRC

SEQ ID NO: 50 - protein, 7 aa, Artificial Sequence
  Synthetic polypeptide
CSVGRLK

SEQ ID NO: 51 - protein, 5 aa, Artificial Sequence
  Synthetic polypeptide
CHQDF

SEQ ID NO: 52 - protein, 9 aa, Artificial Sequence
  Synthetic polypeptide
CSFDEANPC

SEQ ID NO: 53 - protein, 5 aa, Artificial Sequence
  Synthetic polypeptide
CRNRA

SEQ ID NO: 54 - protein, 9 aa, Artificial Sequence
  Synthetic polypeptide
CVSDRKVAC

SEQ ID NO: 55 - protein, 9 aa, Artificial Sequence
  Synthetic polypeptide
CKRGRFAKL

SEQ ID NO: 56 - protein, 7 aa, Artificial Sequence
  Synthetic polypeptide
CAQPNSR

SEQ ID NO: 57 - protein, 9 aa, Artificial Sequence
  Synthetic polypeptide
CRPTRRVSC

SEQ ID NO: 58 - protein, 9 aa, Artificial Sequence
  Synthetic polypeptide
CRNGLNKRC

SEQ ID NO: 59 - protein, 6 aa, Artificial Sequence
  Synthetic polypeptide
CGFRSD

SEQ ID NO: 60 - protein, 9 aa, Artificial Sequence
  Synthetic polypeptide
CRKTVGPRC

SEQ ID NO: 61 - protein, 9 aa, Artificial Sequence
  Synthetic polypeptide
CEVMQRKRC

SEQ ID NO: 62 - protein, 9 aa, Artificial Sequence
  Synthetic polypeptide
CVASVKRKC

SEQ ID NO: 63 - protein, 5 aa, Artificial Sequence
  Synthetic polypeptide
CDANQ

SEQ ID NO: 64 - protein, 9 aa, Artificial Sequence
  Synthetic polypeptide
CRRTAIKKC

SEQ ID NO: 65 - protein, 9 aa, Artificial Sequence
  Synthetic polypeptide
CLSKRTPRC

SEQ ID NO: 66 - protein, 9 aa, Artificial Sequence
  Synthetic polypeptide
CVDSEATDC

SEQ ID NO: 67 - protein, 9 aa, Artificial Sequence
  Synthetic polypeptide
CPRTAKVLC

SEQ ID NO: 68 - protein, 9 aa, Artificial Sequence
  Synthetic polypeptide
CQSRSPRNC

SEQ ID NO: 69 - protein, 9 aa, Artificial Sequence
  Synthetic polypeptide
CNKNGTAPC

SEQ ID NO: 70 - protein, 9 aa, Artificial Sequence
  Synthetic polypeptide
CTDRHSTNC

SEQ ID NO: 71 - protein, 9 aa, Artificial Sequence
  Synthetic polypeptide
CDALAPNSC

SEQ ID NO: 72 - protein, 9 aa, Artificial Sequence
  Synthetic polypeptide
CIDGRTDLC

SEQ ID NO: 73 - protein, 9 aa, Artificial Sequence
  Synthetic polypeptide
CMNVESSPC

SEQ ID NO: 74 - protein, 9 aa, Artificial Sequence
  Synthetic polypeptide
CREKNSQRC

SEQ ID NO: 75 - protein, 9 aa, Artificial Sequence
  Synthetic polypeptide
CLVRPERKC

SEQ ID NO: 76 - protein, 9 aa, Artificial Sequence
  Synthetic polypeptide
CRKRMNRTC

SEQ ID NO: 77 - protein, 9 aa, Artificial Sequence
  Synthetic polypeptide
CVDITSPDC

SEQ ID NO: 78 - protein, 9 aa, Artificial Sequence
  Synthetic polypeptide
CSYEKEPVC